European Patent Application EP 4 659 810 A1, published December 10, 2025. Title: BKV NEUTRALIZING ANTIBODIES. Applicant: Université de Strasbourg. The sequence listing filed with the application follows.

SEQUENCE LISTING (43 sequences)

SEQ ID NO: 1 - protein, 8 aa, synthetic construct
  VARIANT 3: note = X is S, T or N
  VARIANT 4: note = X is F, I or L
  VARIANT 6: note = X is S or G
  VARIANT 8: note = X is A or G
GFXXRXYX

SEQ ID NO: 2 - protein, 16 aa, synthetic construct
  VARIANT 2: note = X is K or R
  VARIANT 5: note = X is G, D or N
  VARIANT 6: note = X is V or A
  VARIANT 14: note = X is I, F or L
AXDRXXZWLGSEPXDP

SEQ ID NO: 3 - protein, 9 aa, synthetic construct
  VARIANT 6: note = X is S or P
QQYGSXPRS

SEQ ID NO: 4 - protein, 123 aa, synthetic construct
  VARIANT 10: note = X is G or A
  VARIANT 23: note = X is A or V
  VARIANT 28: note = X is S, T or N
  VARIANT 29: note = X is F, I or L
  VARIANT 31: note = X is S or G
  VARIANT 33: note = X is A or G
  VARIANT 43: note = X is K or R
  VARIANT 52: note = X is N, T, S or R
  VARIANT 54: note = X is A, S or N
  VARIANT 56: note = X is V, A or T
  VARIANT 57: note = X is S or T
  VARIANT 58: note = X is T or A
  VARIANT 62: note = X is E or D
  VARIANT 75: note = X is S or F
  VARIANT 79: note = X is L or M
  VARIANT 80: note = X is Y or F
  VARIANT 84: note = X is N, H or D
  VARIANT 98: note = X is K or R
  VARIANT 101: note = X is G, D or N
  VARIANT 102: note = X is V or A
  VARIANT 110: note = X is I, F or L
  VARIANT 118: note = X is L or M
EVQLLESGGXLVQPGGSLRLSCXASGFXXRXYXMNWVRQAPGXGLEWVSSLXSXGXXXYYAXSVKGRFTISRDNXKNTXXLQMXSLRGEDTAVYYCAXDRXXZWLGSEPXDPWGQGTXVTVSS

SEQ ID NO: 5 - protein, 108 aa, synthetic construct
  VARIANT 28: note = X is R or S
  VARIANT 29: note = X is V or L
  VARIANT 30: note = X is S or G
  VARIANT 31: note = X is S or N
  VARIANT 32: note = X is N or S
  VARIANT 41: note = X is P or F
  VARIANT 43: note = X is Q or L
  VARIANT 20: note = X is R, G or D
  VARIANT 54: note = X is S or R
  VARIANT 57: note = X is T or I
  VARIANT 67: note = X is G or E
  VARIANT 95: note = X is S or P
EIVLTQSPGTLSLSPGERATLSCRASQXXXXXYLAWYQHKXGXAPRLLIYXASXRAXGIPDRFSGSXSGTDFTLTISRLEPEDFAVYYCQQYGSXPRSFGQGTKLEIK

SEQ ID NO: 6 - protein, 8 aa, Homo sapiens
GFSFRSYA

SEQ ID NO: 7 - protein, 8 aa, Homo sapiens
LNSAGVST

SEQ ID NO: 8 - protein, 16 aa, Homo sapiens
AKDRGVEWLGSEPIDP

SEQ ID NO: 9 - protein, 7 aa, Homo sapiens
QRVSSNY

SEQ ID NO: 10 - protein, 9 aa, Homo sapiens
QQYGSSPRS

SEQ ID NO: 11 - protein, 123 aa, Homo sapiens
EVQLLESGGGLVQPGGSLRLSCAASGFSFRSYAMNWVRQAPGKGLEWVSSLNSAGVSTYYAESVKGRFTISRDNSKNTLYLQMNSLRGEDTAVYYCAKDRGVEWLGSEPIDPWGQGTLVTVSS

SEQ ID NO: 12 - protein, 108 aa, Homo sapiens
EIVLTQSPGTLSLSPGERATLSCRASQRVSSNYLAWYQHKPGQAPRLLIYRASSRATGIPDRFSGSGSGTDFTLTISRLEPEDFAVYYCQQYGSSPRSFGQGTKLEIK

SEQ ID NO: 13 - protein, 8 aa, Homo sapiens
GFSIRGYA

SEQ ID NO: 14 - protein, 8 aa, Homo sapiens
LTSNGATT

SEQ ID NO: 15 - protein, 16 aa, Homo sapiens
AKDRDAEWLGSEPFDP

SEQ ID NO: 16 - protein, 7 aa, Homo sapiens
QRVSSSY

SEQ ID NO: 17 - protein, 123 aa, Homo sapiens
EVQLLESGGGLVQPGGSLRLSCVASGFSIRGYAMNWVRQAPGKGLEWVSSLTSNGATTYYADSVKGRFTISRDNSKNTLFLQMHSLRGEDTAVYYCAKDRDAEWLGSEPFDPWGQGTLVTVSS

SEQ ID NO: 18 - protein, 108 aa, Homo sapiens
EIVLTQSPGTLSLSPGERATLSCRASQRVSSSYLAWYQHKFGQAPRLLIYGASRRATGIPDRFSGSGSGTDFTLTISRLEPEDFAVYYCQQYGSSPRSFGQGTKLEIK

SEQ ID NO: 19 - protein, 8 aa, Homo sapiens
GFNFRSYG

SEQ ID NO: 20 - protein, 8 aa, Homo sapiens
LRSSGVTT

SEQ ID NO: 21 - protein, 7 aa, Homo sapiens
QSLSNSY

SEQ ID NO: 22 - protein, 9 aa, Homo sapiens
QQYGSPPRS

SEQ ID NO: 23 - protein, 123 aa, Homo sapiens
EVQLLESGGGLVQPGGSLRLSCAASGFNFRSYGMNWVRQAPGKGLEWVSSLRSSGVTTYYADSVKGRFTISRDNSKNTLYLQMNSLRGEDTAVYYCAKDRDAEWLGSEPFDPWGQGTLVTVSS

SEQ ID NO: 24 - protein, 108 aa, Homo sapiens
EIVLTQSPGTLSLSPGERATLSCRASQSLSNSYLAWYQHKPGLAPRLLIYDASSRATGIPDRFSGSESGTDFTLTISRLEPEDFAVYYCQQYGSPPRSFGQGTKLEIK

SEQ ID NO: 25 - protein, 8 aa, Homo sapiens
GFSFRSYG

SEQ ID NO: 26 - protein, 123 aa, Homo sapiens
EVQLLESGGGLVQPGGSLRLSCAASGFSFRSYGMNWVRQAPGKGLEWVSSLRSSGVTTYYADSVKGRFTISRDNSKNTLYLQMNSLRGEDTAVYYCAKDRDAEWLGSEPFDPWGQGTLVTVSS

SEQ ID NO: 27 - protein, 108 aa, Homo sapiens
EIVLTQSPGTLSLSPGERATLSCRASQSLSNSYLAWYQHKPGQAPRLLIYDASSRATGIPDRFSGSGSGTDFTLTISRLEPEDFAVYYCQQYGSPPRSFGQGTKLEIK

SEQ ID NO: 28 - protein, 8 aa, Homo sapiens
GFSLRGYA

SEQ ID NO: 29 - protein, 8 aa, Homo sapiens
LTSNGATA

SEQ ID NO: 30 - protein, 16 aa, Homo sapiens
ARDRDAEWLGSEPFDP

SEQ ID NO: 31 - protein, 7 aa, Homo sapiens
QSVSSSY

SEQ ID NO: 32 - protein, 123 aa, Homo sapiens
EVQLLESGGGLVQPGGSLRLSCVASGFSLRGYAMNWVRQAPGRGLEWVSSLTSNGATAYYADSVKGRFTISRDNFKNTLYLQMHSLRGEDTAVYYCARDRDAEWLGSEPFDPWGQGTMVTVSS

SEQ ID NO: 33 - protein, 108 aa, Homo sapiens
EIVLTQSPGTLSLSPGERATLSCRASQSVSSSYLAWYQHKPGQAPRLLIYGASSRAIGIPDRFSGSGSGTDFTLTISRLEPEDFAVYYCQQYGSSPRSFGQGTKLEIK

SEQ ID NO: 34 - protein, 8 aa, Homo sapiens
GFTFRSYA

SEQ ID NO: 35 - protein, 8 aa, Homo sapiens
LSSSGTTT

SEQ ID NO: 36 - protein, 16 aa, Homo sapiens
AKDRNAQWLGSEPLDP

SEQ ID NO: 37 - protein, 7 aa, Homo sapiens
QRVGSNY

SEQ ID NO: 38 - protein, 123 aa, Homo sapiens
EVQLLESGGALVQPGGSLRLSCAASGFTFRSYAMNWVRQAPGKGLEWVSSLSSSGTTTYYADSVKGRFTISRDNSKNTMYLQMDSLRGEDTAVYYCAKDRNAQWLGSEPLDPWGQGTLVTVSS

SEQ ID NO: 39 - protein, 108 aa, Homo sapiens
EIVLTQSPGTLSLSPGERATLSCRASQRVGSNYLAWYQHKPGQAPRLLIYGASSRATGIPDRFSGSGSGTDFTLTISRLEPEDFAVYYCQQYGSSPRSFGQGTKLEIK

SEQ ID NO: 40 - protein, 362 aa, Homo sapiens
MAPTKRKGECPGAAPKKPKEPVQVPKLLIKGGVEVLEVKTGVDAITEVECFLNPEMGDPDENLRGFSLKLSAENDFSSDSPERKMLPCYSTARIPLPNLNEDLTCGNLLMWEAVTVQTEVIGITSMLNLHAGSQKVHEHGGGKPIQGSNFHFFAVGGEPLEMQGVLMNYRSKYPDGTITPKNPTAQSQVMNTDHKAYLDKNNAYPVECWVPDPSRNENARYFGTFTGGENVPPVLHVTNTATTVLLDEQGVGPLCKADSLYVSAADICGLFTNSSGTQQWRGLARYFKIRLRKRSVKNPYPISFLLSDLINRRTQRVDGQPMYGMESQVEEVRVFDGTERLPGDPDMIRYIDKQGQLQTKML

SEQ ID NO: 41 - protein, 362 aa, Homo sapiens
MAPTKRKGECPGAAPKKPKEPVQVPKLLIKGGVEVLEVKTGVDAITEVECFLNPEMGDPDDNLRGYSLKLTAENAFDSDSPDKKMLPCYSTARIPLPNLNEDLTCGNLLMWEAVTVKTEVIGITSMLNLHAGSQKVHENGGGKPVQGSNFHFFAVGGDPLEMQGVLMNYRTKYPQGTITPKNPTAQSQVMNTDHKAYLDKNNAYPVECWIPDPSRNENTRYFGTYTGGENVPPVLHVTNTATTVLLDEQGVGPLCKADSLYVSAADICGLFTNSSGTQQWRGLARYFKIRLRKRSVKNPYPISFLLSDLINRRTQKVDGQPMYGMESQVEEVRVFDGTEQLPGDPDMIRYIDRQGQLQTKMV

SEQ ID NO: 42 - protein, 362 aa, Homo sapiens
MAPTKRKGECPGAAPKKPKEPVQVPKLLIKGGVEVLEVKTGVDAITEVECFLNPEMGDPDNDLRGYSLRLTAETAFDSDSPDRKMLPCYSTARIPLPNLNEDLTCGNLLMWEAVTVKTEVIGITSMLNLHAGSQKVHENGGGKPIQGSNFHFFAVGGDPLEMQGVLMNYRTKYPEGTVTPKNPTAQSQVMNTDHKAYLDKNNAYPVECWIPDPSRNENTRYFGTYTGGENVPPVLHVTNTATTVLLDEQGVGPLCKADSLYVSAADICGLFTNSSGTQQWRGLPRYFKIRLRKRSVKNPYPISFLLSDLINRRTQRVDGQPMYGMESQVEEVRVFDGTEQLPGDPDMIRYIDRQGQLQTKMV

SEQ ID NO: 43 - protein, 354 aa, Homo sapiens
MAPTKRKGERKDPVQVPKLLIRGGVEVLEVKTGVDSITEVECFLTPEMGDPDEHLRGFSKSISISDTFESDSPNRDMLPCYSVARIPLPNLNEDLTCGNILMWEAVTLKTEVIGVTSLMNVHSNGQATHDNGAGKPVQGTSFHFFSVGGEALELQGVLFNYRTKYPDGTIFPKNATVQSQVMNTEHKAYLDKNKAYPVECWVPDPTRNENTRYFGTLTGGENVPPVLHITNTATTVLLDEFGVGPLCKGDNLYLSAVDVCGMFTNRSGSQQWRGLSRYFKVQLRKRRVKNPYPISFLLTDLINRRTPRVDGQPMYGMDAQVEEVRVFEGTEELPGDPDMMRYVDKYGQLQTKML